European Patent Application EP 4 696 780 A1, published February 18, 2026. Title: ビフィドバクテリウム属細菌の形質転換方法. Applicant: 株式会社ヤクルト本社. The sequence listing filed with the application follows.

SEQUENCE LISTING (73 sequences)

SEQ ID NO: 1 - DNA, 777 bp, Bifidobacterium pseudocatenulatum
  source 1..777: mol_type = genomic DNA
atgggcaatgtggtggttatcgactccgtggtggcaggagtgggcacgagcactctggccgccttactggcccgcgagctgagcgaacgcggcctcaaatgtgtgctcgtcgacgccgatctgcaaggaggtgggctggatgtgcttcttggcgtggaaaacgaagacggctcacgcttcggggaaatcagcgctccgcttggcaatatcgacggcaaagcgctactgcgggagctgccaatctgggatggtgtgccattgctggcatgcgatccttggaaaaccgaaaatccgcaatcgtgggaagtgcaagcgtgcattcatgcgctatcgcaggtgcgaagcgtggtcgtcgtcgatatggggcaatggaacggactgcaggatttgacggaactgcgcaaggccatccgcattaccgtggtcgaactgacggtacttggtcttgcgcgggccaaagcgaatctgcgggcgcattacggttcgatcggagaacacgatgccgcaacgcaggaacgggagtttctcgtaggcgtgcaaccgcgcggaaccgtacgcgaccatggcacgacggcaatcgaggaagcggcggaatacctcgactgcgatatcaccgcggtcatcaaaccggatgccaagctttgcagcgaactcttggaagggcttggactgcgcacacccaatcgtacgaacgcgaaagccatcgcaacgttggcggatctcattcaggaagcgttgggagaaaagagcatcagtcatggaactcgggccacttag

SEQ ID NO: 2 - DNA, 990 bp, Bifidobacterium pseudocatenulatum
  source 1..990: mol_type = genomic DNA
atggaactcgggccacttagcgatatcgcatccgagccgggcgtcaccgacatcgcggtaacctgcgacggaacggtgtgggtggatcgcggccaaggtatgcggccacatgcattgcgcgtgccattcagcggtccccaagccatccgcgatttcgccgtgcggctgtgctcgcagcttggcagaaggctcgacgacgcctgcccgatagccgacgcgtccacggtggaaggcgtgcgcgtgcacgcggttatcgcaccgctcgttccgcaaggcgccgccatcagcatacgattgccggacgttgttgcgcccagtctggaatctttggcggaaaacggcatgtttccaagcggatggatgcctttgctggaaggattcgtggaacgaagggccagcgtgctcgtgaccggcggaaccggagcaggcaaaaccacgctgctcaaagcaatgcttatgcgatgcgcgccgggggagcgcgtcatcaccgtggaggaggtgcgcgaacttggcatgctcaaccatgccaaccacgtgtcgctggtgacgcgcggcgccaacatggaaggcaaaggcgccatagggctgtcgcagctgatatgcgcgacgttgcgtatgcggccggaccgcattgtggtgggcgaatgcaggggcggcgaaatcgtggatctgctgcgcgcgctgaattccgggcatcgcggaggcatgaccaccttgcatgccaatcaggtgacggcggttccctcacgtttggtggccttgggattgctctccgggctgaatccgcaagccaccgcggcgctcgcgcaagacgcgttcgacgtagtgctgcatgtgggccgagtgggaggcaggcggcgcatcgcgcaaataggacggcttgaattcgcagaggggaaactgcggggaaacctattggccgggtggaacggcagccaaatgcgggcttcgcaacagtggcctgatttcgtgcgcgtatggagtcgttga

SEQ ID NO: 3 - DNA, 732 bp, Bifidobacterium pseudocatenulatum
  source 1..732: mol_type = genomic DNA
atggaaagcctcagcattatttgcgcggtattgtgcggactggccgtatggctgtggcctcgccgaaacgtatgcgatgtgggcgaacgggcgggaaacgtagtggggcgcgcaggcgaaagccttgatgaaaaacctgatggaggattcggcgggcggtctgacggaatcgaagaggcgaacatgccgacgaaaccattgcccgccatcggatgtgtggcgtgcgtggcttccctccgcgcatccgtgcgcagcggagccacattggtgcaggcgttcgaagaattgggtggaacgccgttcgccacacccgaacttaccaggcttcgcataaccatggtgatccgcagccgatgcccgcccaaagagcaatgcggccaagtcgaacggctgagcggcgagctatatgcggcctgtcagctgagcctgacgctcggatgcgaaaccggccgatgcctgcaggcggtggctgaatcgttgaaacggcaacgattattggatgatctgcgtaccaacgcattcgccatgcccaaagcgacggtgaaactcctgatggcgttgccgctgctcactgtgctcttgggagaaggtatgggtgcgcactcattggccttccttgtttcaggggtcaaaggcttggcatgcctcggatttgccctctgttgctacacgttcggacttatctggatacgtgcgctgatgcggcaggatgatatgaaaggagccatgtga

SEQ ID NO: 4 - DNA, 525 bp, Bifidobacterium pseudocatenulatum
  source 1..525: mol_type = genomic DNA
atgactggcttatggatgctgacggcggcggtgtgcgcggccgaagcgatgtggctgaagcagtggaggccggtccgtgtgccagccgaccttgcgcccgccggacgagtgcgggaacttccgctgccgctggtattggagatgctcagcgtcgccatacggcagggatcctccattccacgcgcgctgattgccgtgggcgatatcgctgcgggagaattcggcgcgggactacggtcggccggagaacagttgaacaaaggtgtttcctgggatgatgcgtggccagatgatggcgatcttgcggtggtgcgcgatgcgttcgcctcgtcatggcacagtggcgcctcgccggtggaacgtttggaaacagcggtcgaacaattggattgggatgagcgctcgcagatcgaacaggctgcagcgaaattgtcggttcgtttgttgctaccgaccggattgtgctttcttcccgcatttgttgcggtggggattattccggccgttatgtcgtttgtgggatga

SEQ ID NO: 5 - DNA, 288 bp, Bifidobacterium pseudocatenulatum
  source 1..288: mol_type = genomic DNA
atgaacaacgaaacgccaatcaacgtcgatggctcgccagacctgatgggcaaggcaggacagctgctgcatgccatgcgtgaacgggccggcaaagcggtatgcctgctggacgcgcgtatgcgcacgctgaccgtcgaaccggaggaaggcgctgccactgccgaatatgcggtggttttggttgccgccaccggattcgcagccgttttggtgggcattatgaaatccgatgccatcaaaacgctgctgaccaacatcatcaagaaagcgctgagcgtcgggtga

SEQ ID NO: 6 - DNA, 369 bp, Bifidobacterium pseudocatenulatum
  source 1..369: mol_type = genomic DNA
atgctgaggcaatggtggaaacgccataccgatgatgccgatgagggagcggccaccgcggaattcgcggtggtgctcccctgcgtggcggcggtggcgattttggtgttgtgcttggggcatgcgtctgtggtgtccatgaattgccaggatgcggcggcggccggtgccagggctttcgcggttgatgatacgggcggcgaatcgaaggcgaggaccgcggtcatggcggctgcgggaggttcggcgacggtacggttcgagcgtggggcggacttcgtcaccgtcacggtgcaatgccctgtggtgccggatccgaccggtgtgctgcccactcgagttaccggcaaggcgacccgctacttctag

SEQ ID NO: 7 - DNA, 390 bp, Bifidobacterium pseudocatenulatum
  source 1..390: mol_type = genomic DNA
atggataatgtgaaacgccttgtgaaacattggtttgcttggattcgcgggtccgatgagggttcggggaccatatccggtgtggctttgatcgcagtggccgccatcatgctgggcgcggccgcgtcggcgggcaatctgctgctgtgcttgcatcgcgcgcagaatgcggccgacctggcgtcggtagcggcggccaatgcgttgtattcgggatcgtccgatccttgttccgtggcggaacgcactatatccggcaataatgcgacgatcggatcctgcacgatagaaggcgaggatgtgctggtcgaagcgcaggtcggcacgcaaatgccattcgtatcgcatgtcggcaaacagtcacgggcggggccgattgtctgcgaataa

SEQ ID NO: 8 - DNA, 1371 bp, Bifidobacterium pseudocatenulatum
  source 1..1371: mol_type = genomic DNA
atgaacgagaacacaaccgccgatacgagcgtcaacgcaaccgccatcgacgatgagaccctgtcacgcgcggtgctcacctattgtctggacagcgccgatgcgatgatgtacgcgctggtcaaaggcatcggatcagccacgcataccctgcaactgcttgccgacagcggtccgggcaatcatgaaagcgtggccacggcagcctataaaaccttggacgcggcgctcatcaacggcattacacgttggggacgcaccatcaatgctcgaggtatggcctccttccacggcgcaatggtctcgtggcagcatcgcctgaccacattgcccagcaccgaccccgaggagctcaaaacgtggttcaccgcaaacggcacgcagtggatcgtcgcgccgcatcacccctactggccttcgcagcttgccgacctcaccatacacacggactgggccgcgccattatgcctatgggggaaaggtgacccccaagcgttggtgtcatgctccgaaccggtcggtgtcgtcggatcacgcggcgtaagcgagtacggaaggcaaagcgcacacgagctcgccaaacaagcggcccgagcaggccatctcatagtgtcaggaggcgctctgggcaccgatgcggccgcccactggggagccatccaagccatggacgagatcggaacgcccctcgcaggacgcaccgtcgcggtattcgccggaggactcaaccatatcggtccgaaaagcaacgagcgcctcttcgaaaccatcatcaaccattccggcgcgctcatctcggaactctgccccggaaccgttccggaagccagacgattccttatcaggaaccgcctgatagcggcgctatcatccaccctcatcgtagcccaggcacgcgcacgctccggcgcgcttaacaccgcaggatgggccaacgaactcaaccgccgtgtattcgccgtgccaggagatgtaaccatgcctcacaacacaggatgcaaccgactcatacaagaaggccaagcctccatcatctgctcgctgaccgatatcgacgaattctgccacgcagcgcatcgcccgcaatcagccgacgcggcagacaacgacgacgaaccgtcggaagagtcaaccgacaccagtctgtcgcaaccaaccaacgccactgcagccatactcaaagccatacgaacatgcagcgcgaaatacggccacgtctccactgacggtctactcgccatcctggccgaaagcaatcccggagaatactcaatctcacgaatcagcatggagctgggattaatggaactcaacggacttatctgcacacagcatggcaacatcaccatcaccgacgcaagcgccacatga

SEQ ID NO: 9 - DNA, 1530 bp, Bifidobacterium pseudocatenulatum
  source 1..1530: mol_type = genomic DNA
atggctatcggcagcgcgctttccgtgggtctcatcggcctgaaagccttcatcatccaaatccaggcgttcgtatctccgggactcccctacttttccatcatcggacttcccgacacctcgctctccgaagcgagggaacgtgtcaaatccgcatgtcaggccagcggtgccaaatggccggaaacacgggttacagtcaatctttcgccggcgtccatgcccaaacgcggatcctcacacgatctggcgatcgcagcgagcgtgcttagcgcatccggaacgataccgcatgactgcttgaacgacaccgtcgtgctcggagaggtgaatctcgatggcacggtactgcccatcaacggtctgctgccgattctgctgcatgcacgcgatcaaggcgtatgcaaggtgatcgtaccgcatgccaatttggacgaggcggcccttgtgcccgacgtcgacgccattgggatacgtcacgtcggcgaactgatcgaactgatgggaggcaccgcgaactatacgatacccgatatgatccgagacgtggatgccaacgacggcgccatgtcggtatgtcctcctcccggagatatgaacgaagtcatggggcaggaaacggccaaatgggcgttggaagtggcggctgccggcggccatcatctgatgatgaccggtcctcccggcaccggaaaaaccatgctcgcctcgcgcattcccggcattatgagtccgctcagcgaatcggaacaactggaagtcgcctcgatccgctccctatgcggcacattgcccagctatggcatcagcgatgttccgccattcgaagcaccgcaccataccgcatccaccgcatccttggtcggcggcggcgcgggattggctcaaccaggcgcgatcacgcgggcgcatcggggcatcctattcatggacgaggcgcccgaattctcggcacgcaccctgcaaaccttgcgcgaaccattggaatccgggtatgtggcgatatcccgcgcgaaaggcaccacctactatccggcacgattccaactgatcatggcggccaatccttgcccctgcggctatgcatacggcaacggcgagcgctgcacgtgcagggaaaaagaccgtatcaagtacttcagccgcctgtcggggccgatcctcgaccgcatcgacattcagatcgaagtgcctcctgtggaacgcatcaacccaggcacggttccttccggcgaatccagccacgccatccgcctgcgggtcatggtggcaaggcaaacggcacaggaacgtttccgggaattcggatgggtctgcaatgcgcaagccaccggaacatggcttcgcgccaacacgtccacaaaagccatcgagctcgtgaaccatgcgttggccagcgaacggctcagcctcagaggggcggaccgagccatgcgactcgcatggacgctatccgacctgtcaggcaaaacctctcccggaccggaagagatgatgcaaggaatctccatgagaacgaggttgacatga

SEQ ID NO: 10 - DNA, 453 bp, Bifidobacterium pseudocatenulatum
  source 1..453: mol_type = genomic DNA
atgaacggcaacacaacacataacgttccgaacgcaacgcagcgctcggaacagcttcttgattccatcgcacggcgactgcatgatggcacactgtgcgcacgacaggtcggcgaactcggcgaacagtatgcggccgcatggctggaaagacaaggctggcagacgctcgaccgcaactggcactgccgatatggcgaactcgatatcgtttcacgcgacgatacgggattcatcgtcttcgtcgaagtcaaaaccaggcggacgctccgctatggcactccgcaggaagccgtgacgtcatccaagcagatcaacctgcgccacgcggccgtgcaatggctgtcggacagcgaccatcgcacgccacataacggcgtgcgcttcgacgtcgtcaccgtcatcgtccgtgatggcaaaccgcttgtccaccatatcgaaggagcgttctga

SEQ ID NO: 11 - DNA, 792 bp, Bifidobacterium pseudocatenulatum
  source 1..792: mol_type = genomic DNA
atgggcattatcgttaccccgccgggcaggcgcaacaggcaagccgaaaccgcatcgcagtccgcgcaacggctgcgcggacttggcatgcccgaaacacgtggaaagaacgcgcgcgggcagaacgttcgcaacgaacatgctgttcccgcgatatccgaaacaacctcaatatccgagatttccgcagcggctgaaacgtccactgcaatcgcgacaactgaacaatcgcctgaacccgcaaaacccacattgcgggatctggccggcgtcaagccttccgacaaaccgactgaacaggaccggcccaaacgcgaccgtccacgactcgtcttccaaccaatccacgcggtcatcgccatactcaccctgtcgtgcgcgctctgcgcaagcctgaccatgctcatccaacaggccgtccactacagtgcgctccaacaatcgcagatcacccaatccgaacaatcgaaggcgaacggaaccgagaaagacaagacggcgtccacgcaaacaacaccaagccagcagccatccacggaacccgacagccagagcgaaccaacatccggaccagcggagcccgccgatccggctgacggtctgctgaacatcaacaccgcaggatccgacgaactgcagaccttgaaaggcgtcggccccgtgaccgcgcaacgcatcatcgactatcgcaatcagatcggccgtttcgacaatgtcgaccaactgttggaagtcaaaggcatcggcgagaaaacgctggcgaaattccgagaccaagtgtgcgcacgatga

SEQ ID NO: 12 - DNA, 1752 bp, Bifidobacterium pseudocatenulatum
  source 1..1752: mol_type = genomic DNA
atgagaggaaacacgttcgaatggcgggatggggagcaggggagcagggattggcgtctgctgccggccgccctatgcgggtgggcggcgagcttggccacgcatatgggattcgactattgcgtcgaacgggatggtcggttcggcatgctgccgctcgttgtggcattggcggtaccgttgctggcattattgggattattgggattgccgttcctgcgatcgcctatgctgcgagtgccggttggcgtgcggcgggcggtctcggcatggcatttcagcattatcgtatgcgtggtcgcggcgatggcatgcgcgtcttccgcgttgacctacgacgtattgcaatggagggatgcggcctcgtacgcggccagaaacggcgaaagcgacgttgtcacgctggtacgtacgacatctcccgcagtgaattcgaacagacgtgcaaacgattgccagattgatgcgacgatctcaacgatcacggcaagccaggtcacgcagccaagcatgatgcgggtgcgcgtctatgcggaccggccggactgcggcacgctcaaacaaggcggcgaataccggatgcggggcacgctcgccatatcgcaatacggtgccatgccgctatggctgacggacatcgcctccgtggaacgcatacggggaccgaacctcgcattgcgcacgatcggcatgatgcagcaggcgttcttcgaacagacgtcacggctttccgaccaagggaaagtgctcgttcccggcctgaccttaggtattcttgggcaggattacgttcctccagatagtggcaatggccagacgggcacgggtattgattccacatacgccaatctgcttgaaaacgccttccaacgttcgggcatactgcatctgatggcggtcagcggcgggcatcttgcggtcgtcgccaccctggtgcgcgccgtctgctcgttcctgctgctgcccaaacgcgtcacggccatcgccatcggcgcgtcgtacatcatgctggcgatgtgcgtgttcccatccgattcggtgtcgcgcgccctgctcatgggtttggcgggagcgggcttcctgttcctcggccgaagaacgcaagccctgtcaaccctcagctggaccacgttgggcatgctcatggtcaatccgcacatgtcacgcagtttcggattcgcattgtcatgcgccgccgtacttggcatcgtactgttcgcaggaccgttaggcgcatggctcacaccgatcatgccggcattcatcgcgcaaaccatggccatgaccatcgccgcgcaactcttcaccctgccgatccaagtgcttatcgaaccagaactgccggtctactccattccagccaatctggtcgtcgcacccttcgtgggattctccacacttgccggactcgccagtctcgccatctcatggatacttccaagcctcgggttcatattcgccagcctcgcctcatggggcaccgccatcatggaattcatggccctcaacctcggatcaggagaccacgccaccattccatggaccggagacgcaggcggcgcgctactgatcatcctcgtcgaaatcatcggatacacgaccgcacgattcgccggaacactcttcgcccgcatcaccacaacggaaccaaacctgccgggccgacgcctcatacacaatccgatcgaacgggcgaaagcatggggcgaacgaacctacaacgcgctcaagaccatgaaatggaacgaatga

SEQ ID NO: 13 - DNA, 642 bp, Bifidobacterium pseudocatenulatum
  source 1..642: mol_type = genomic DNA
atggatattcatgttttgaaccacccgctggtggaccacaagctcaccgttcttcgcgacaagaacaccccgtcctccacgttccgcgagctcgtttccgaactcgtgatgcttgaggcctacgaggccacccgcgacgtcgaagtcgtggacaagccgatcgagacccccgtcgctccgatggtaggcaagcacatcgcttccccggcgccgatcattgtgcctgtgctgcgcgctggcctgggcatgcttgacggcatgaccaagatgatcccgtccgctgaggtcggcttccttggcatgaagcgcgacgaggagaacccaacccagcagatcacgtacgcgaaccgtctgcccgacgatctgagcggccgtcagtgcttcctgatcgacccgatgctcgccactggcggcacgctggtcgcagcaacacattacctggccgagcgcggcgcaaaggatgttaccgccgtgtgcattctgggcgctccggaaggcctgaagttcgttgaggagaacctcgacccatccattaagttcaagctggtgctgtgcgccgtcgacgagaagctcaacgacaagtgctacatcgtgccaggcttgggcgatgccggcgaccgtctatatggcgtgatcgactga

SEQ ID NO: 14 - DNA, 2091 bp, Bifidobacterium pseudocatenulatum
  source 1..2091: mol_type = genomic DNA
atggctgactcactcgcatcgcagatcatcactgcaatcggtggtcctgaaaacgttcgcagtctgacgcattgcgccactcgactgcgctttgaactggttgacgcatccaaggtcgatcagaatagtctcgagcacatgcagggcgtgctcggcgcggtgccgcagagcggcgaccgcttccaggtggtcatcggcggtggcgttgccaccgtgtacgaaaacatcatgcatctgcccgaaatggccggtgtcggcggtgcctccgcatccgacgatggtcagaagagcaatgccgacgtcaaggccgaagcccgttccaaggcccgcggcaaggtggcttggctggactccttcttcgagtatctctccgattccttccgcccgattctgggcgtgctgctcggcgcttccatcatcatcgcgctggtcaacctgcttatttcgctgaacgtcattccgaatgacgaggtttccgcaggctgggtattcgtgaaagccatctggaagggcgtattctacttcctgccgatcatggtcgcctacaacgcgtccaagaagctcaaagtcgacccatggctgggtggtgccatcatggccatgctcatgaccccgcagttcaccggcttgatggacgccaagaccaccacgtgcgtggagaacgccgctctgggcaccaagtcttgcatggccaacatattcggtctgccgatggcattgagcgactattccggcaacgtgttcgtgccgctgctcatggccgccgtgcttgctctcgtctaccacggattgaagaggatcatcccggaaagcgtccagctggtcttcgtgccgttcttctgcatgatcatcgttggcgcgctgaccgccttcatcatcggcccgatcggcgtgtgggtcggcaacggcctcggcgtcggcttggcctggatgaacacccatgccccgttcatcttcgccatcatcattccgatgctgtacccgttcctcgtgccgctcggtttgcactggccgctcaacgccctgatgctcatgaacatccagactctcggctacgacttcatccaaggcccgatgggcgtgtggaacttcgcctgcttcggcgctaccgctggcgtgctcttccttgctgtgcgtgacaaggataaggacatgcgccagaccgctttgggcgcacttgcggccggcctgctcggtggcgtttccgaaccgtctctgtacggcattcacctgcgttacaagctcatctacaagcgcatgctggtgggctgcggtctcggtggcgtcgtcatcgccatcctcggttggctcttcccgtccgtcaccgccgccggccagaccgtgcatggcgtgaccaccaccgctttcgcattcacctcgttgctgaccattccggtcttcaatcagatgtgggtgtatgcagtgtccatcgccgtgtccttcctcacctccttccttctgatcatcaccttcgactaccgcactccggaacagaaggccgaagtgctggcccgtgcggctgccaatcagaagaccgctgtctcgtcggtcgaagccaagggagtcgctccggctgctgccaccgcgactgccactgttgccgccaccaagactgaagccccggctgctgctgccaccaccaccgtggtgaacgctccagtcgcaggccatgtgatttccctggatgaaaccggcgatccggtgttcgcatcccgcgcactaggcgaaggcgtcggcatccagccggcagacagcaccgtcgtcgcgccggtatccggcgtgctgcagaccgtcgccgaaaccggtcacgcattcggcatcaaaaccgatgatggcgcggaagtgctcgtgcacgtcggcatcgacacggtgaagatgaacggcgaaggcttcgatgtgaaggtcaaggccaacgaacacgtgaacgcgggggacaacctcgttgtcgtcgactttgataaggttaaggaagctggatacagcaccaccacattgatgacggtgctgaacacagtggccttcgcgtccgtcacgccaaagaccggcgtcgacgtcaaggccggtgagtcggtgatcgacattcagcgctga

SEQ ID NO: 15 - DNA, 21 bp, synthetic construct
  source 1..21: mol_type = other DNA
gggcaagatcggcatcatcta

SEQ ID NO: 16 - DNA, 21 bp, synthetic construct
  source 1..21: mol_type = other DNA
cacattggtggtgttcacgtc

SEQ ID NO: 17 - DNA, 22 bp, synthetic construct
  source 1..22: mol_type = other DNA
cgagaatgcgaacacgtacttc

SEQ ID NO: 18 - DNA, 22 bp, synthetic construct
  source 1..22: mol_type = other DNA
ctgctcggtgttgtaatcgttg

SEQ ID NO: 19 - DNA, 28 bp, synthetic construct
  source 1..28: mol_type = other DNA
tcctgtggatttcgacggtgacgagcag

SEQ ID NO: 20 - DNA, 28 bp, synthetic construct
  source 1..28: mol_type = other DNA
gagtgcggttgatggtgcatacggcaag

SEQ ID NO: 21 - DNA, 21 bp, synthetic construct
  source 1..21: mol_type = other DNA
aagtgtggttttgtccgttcg

SEQ ID NO: 22 - DNA, 35 bp, synthetic construct
  source 1..35: mol_type = other DNA
tagatgtgccgaaatcgggacttggtacttttcgg

SEQ ID NO: 23 - DNA, 35 bp, synthetic construct
  source 1..35: mol_type = other DNA
taccaagtcccgatttcggcacatctaaaccaagg

SEQ ID NO: 24 - DNA, 35 bp, synthetic construct
  source 1..35: mol_type = other DNA
tagatgtgccgaaaccagtgaatgccctcctgatt

SEQ ID NO: 25 - DNA, 35 bp, synthetic construct
  source 1..35: mol_type = other DNA
gggcattcactggtttcggcacatctaaaccaagg

SEQ ID NO: 26 - DNA, 21 bp, synthetic construct
  source 1..21: mol_type = other DNA
cgcaagtgtgtcgtttctgtt

SEQ ID NO: 27 - DNA, 35 bp, synthetic construct
  source 1..35: mol_type = other DNA
tggcggtgcttccgggttccggtgattccttgttc

SEQ ID NO: 28 - DNA, 35 bp, synthetic construct
  source 1..35: mol_type = other DNA
cacgggcgacgggctgttctaccaacttccacgac

SEQ ID NO: 29 - DNA, 20 bp, synthetic construct
  source 1..20: mol_type = other DNA
gcgttcctgaatgggaagta

SEQ ID NO: 30 - DNA, 35 bp, synthetic construct
  source 1..35: mol_type = other DNA
tttcctcgcgattatggccgcatcagagctcaacc

SEQ ID NO: 31 - DNA, 35 bp, synthetic construct
  source 1..35: mol_type = other DNA
tgagctctgatgcggccataatcgcgaggaaaagc

SEQ ID NO: 32 - DNA, 20 bp, synthetic construct
  source 1..20: mol_type = other DNA
tgaagtaccgttcgttcgtg

SEQ ID NO: 33 - DNA, 20 bp, synthetic construct
  source 1..20: mol_type = other DNA
cgatcattgtgcctgtgctg

SEQ ID NO: 34 - DNA, 20 bp, synthetic construct
  source 1..20: mol_type = other DNA
tgatctgctgggttgggttc

SEQ ID NO: 35 - DNA, 20 bp, synthetic construct
  source 1..20: mol_type = other DNA
gacaattccaagtggggttc

SEQ ID NO: 36 - DNA, 20 bp, synthetic construct
  source 1..20: mol_type = other DNA
gtcgcggaaaactggagtaa

SEQ ID NO: 37 - DNA, 19 bp, synthetic construct
  source 1..19: mol_type = other DNA
tcatgcacctgaaccgact

SEQ ID NO: 38 - DNA, 35 bp, synthetic construct
  source 1..35: mol_type = other DNA
ttagatgtgccgaaagaaacgagccaaccgtacct

SEQ ID NO: 39 - DNA, 22 bp, synthetic construct
  source 1..22: mol_type = other DNA
tttcggcacatctaaaccaagg

SEQ ID NO: 40 - DNA, 21 bp, synthetic construct
  source 1..21: mol_type = other DNA
ccagtgaatgccctcctgatt

SEQ ID NO: 41 - DNA, 35 bp, synthetic construct
  source 1..35: mol_type = other DNA
gagggcattcactggcacagtgcgatgactggttc

SEQ ID NO: 42 - DNA, 20 bp, synthetic construct
  source 1..20: mol_type = other DNA
gtacgaaatcgtcccgtttg

SEQ ID NO: 43 - DNA, 20 bp, synthetic construct
  source 1..20: mol_type = other DNA
gcttgccgaacttttgctat

SEQ ID NO: 44 - DNA, 20 bp, synthetic construct
  source 1..20: mol_type = other DNA
tctgcacccacctctgtacc

SEQ ID NO: 45 - DNA, 20 bp, synthetic construct
  source 1..20: mol_type = other DNA
ataatggaacggctcaccac

SEQ ID NO: 46 - DNA, 35 bp, synthetic construct
  source 1..35: mol_type = other DNA
caaaagttcggcaagcaagcctgcacagatcaacg

SEQ ID NO: 47 - DNA, 97 bp, synthetic construct
  source 1..97: mol_type = other DNA
agaggtgggtgcagacgtggttatgcgtgtctgatgcgtatgttttcgatggattccgttgatctgtgcaggcttgattcaagtccagcagaaagga

SEQ ID NO: 48 - DNA, 20 bp, synthetic construct
  source 1..20: mol_type = other DNA
gagacgaaggtggtggtgat

SEQ ID NO: 49 - DNA, 21 bp, synthetic construct
  source 1..21: mol_type = other DNA
tcgctgtccccggaaatagtc

SEQ ID NO: 50 - DNA, 21 bp, synthetic construct
  source 1..21: mol_type = other DNA
ctgtcaccgcatccatcaacg

SEQ ID NO: 51 - DNA, 20 bp, synthetic construct
  source 1..20: mol_type = other DNA
catcctggccgaaagcaatc

SEQ ID NO: 52 - DNA, 20 bp, synthetic construct
  source 1..20: mol_type = other DNA
ggtgatgttgccatgctgtg

SEQ ID NO: 53 - DNA, 20 bp, synthetic construct
  source 1..20: mol_type = other DNA
cgcatgactgcttgaacgac

SEQ ID NO: 54 - DNA, 20 bp, synthetic construct
  source 1..20: mol_type = other DNA
cttgcatacgccttgatcgc

SEQ ID NO: 55 - DNA, 20 bp, synthetic construct
  source 1..20: mol_type = other DNA
cgcatggctggaaagacaag

SEQ ID NO: 56 - DNA, 20 bp, synthetic construct
  source 1..20: mol_type = other DNA
cgcctggttttgacttcgac

SEQ ID NO: 57 - DNA, 20 bp, synthetic construct
  source 1..20: mol_type = other DNA
gagacggttcaggtttccag

SEQ ID NO: 58 - DNA, 35 bp, synthetic construct
  source 1..35: mol_type = other DNA
agcaaaagttcggcaagcatcgcagggttcctcca

SEQ ID NO: 59 - DNA, 92 bp, synthetic construct
  source 1..92: mol_type = other DNA
agaggtgggtgcagacctggaacgtatggcatggttgcgcaatgcggtcgcgcatcggtggaggaaccctgcgattggtgcggaacggtaca

SEQ ID NO: 60 - DNA, 21 bp, synthetic construct
  source 1..21: mol_type = other DNA
cgtgtcaaagaagaagcagga

SEQ ID NO: 61 - DNA, 97 bp, synthetic construct
  source 1..97: mol_type = other DNA
agaggtgggtgcagacgtggttatgcgtgtctgatgcgtatgttttcgatggattccgttgatctgtgcaggcttctcgttcatgtcaacctcgttc

SEQ ID NO: 62 - DNA, 20 bp, synthetic construct
  source 1..20: mol_type = other DNA
gatcaaggcgtatgcaaggt

SEQ ID NO: 63 - DNA, 20 bp, synthetic construct
  source 1..20: mol_type = other DNA
ctccatgctgattcgtgaga

SEQ ID NO: 64 - DNA, 35 bp, synthetic construct
  source 1..35: mol_type = other DNA
aaaagttcggcaagcgagaacacaaccgccgatac

SEQ ID NO: 65 - DNA, 96 bp, synthetic construct
  source 1..96: mol_type = other DNA
agaggtgggtgcagatgacagggtctcatcgtcgatggcggttgcgttgacgctcgtatcggcggttgtgttctctcagaacgctccttcgatatg

SEQ ID NO: 66 - DNA, 20 bp, synthetic construct
  source 1..20: mol_type = other DNA
tattccggtttcctcggttc

SEQ ID NO: 67 - DNA, 20 bp, synthetic construct
  source 1..20: mol_type = other DNA
gttgatgcgttccacaggag

SEQ ID NO: 68 - DNA, 35 bp, synthetic construct
  source 1..35: mol_type = other DNA
aaaagttcggcaagcgtccaccatatcgaaggagc

SEQ ID NO: 69 - DNA, 97 bp, synthetic construct
  source 1..97: mol_type = other DNA
agaggtgggtgcagatgagacccacggaaagcgcgctgccgatagccatcagaacgctccttcgatatggtggacgattcaagtccagcagaaagga

SEQ ID NO: 70 - DNA, 20 bp, synthetic construct
  source 1..20: mol_type = other DNA
tactaccgcgacaccaacac

SEQ ID NO: 71 - DNA, 35 bp, synthetic construct
  source 1..35: mol_type = other DNA
aaaagttcggcaagccgaaggatgggagttatcca

SEQ ID NO: 72 - DNA, 95 bp, synthetic construct
  source 1..95: mol_type = other DNA
agaggtgggtgcagaggtgggaaccgtttccgcataaggcgacacgccgaacatgtggataactcccatccttcggtccaccgatacagcgagat

SEQ ID NO: 73 - DNA, 20 bp, synthetic construct
  source 1..20: mol_type = other DNA
tgaggatgatggtgttgtcg